European Patent Application EP 4 759 929 A1, published June 17, 2026. Title: DNA聚合酶突变体及其在测序中的应用. Applicant: 深圳华大智造科技股份有限公司. Application CN. The sequence listing filed with the application follows.

SEQUENCE LISTING (2 sequences)

SEQ ID NO: 1 - protein, 775 aa, synthetic construct
MILDADYITEDGKPIIRIFKKENGEFKVEYDRNFRPYIYALLKDDSQIDEVRKITAERHGKIVRIIDAEKVRKKFLGRPIEVWRLYFEHPQDVPAIRDKIREHSAVIDIFEYDIPFAKRYLIDKGLIPMEGDEELKLLAFAIATLYHEGEEFAKGPIIMISYADEEEAKVITWKKIDLPYVEVVSSEREMIKRFLKVIREKDPDVIITYNGDSFDLPYLVKRAEKLGIKLPLGRDGSEPKMQRLGDMTAVEIKGRIHFDLYHVIRRTINLPTYTLEAVYEAIFGKPKEKVYAHEIAEAWETGKGLERVAKYSMEDAKVTYELGREFFPMEAQLSRLVGQPLWDVSRSSTGNLVEWYLLRKAYERNELAPNKPDEREYERRLRESYAGGYVKEPEKGLWEGLVSLDFRSLYPSIIITHNVSPDTLNREGCREYDVAPEVGHKFCKDFPGFIPSLLKRLLDERQEIKRKMKASKDPIEKKMLDYRQRAIKILANSYYGYYGYAKARWYCKECAESVTAWGREYIEFVRKELEEKFGFKVLYIDTDGLYATIPGAKPEEIKKKALEFVDYINAKLPGLLELEYEGFYVRGFFVTKKKYALIDEEGKIITRGLEIVRRDWSEIAKETQAKVLEAILKHGNVEEAVKIVKEVTEKLSKYEIPPEKLVIYEQITRPLHEYKAIGPHVAVAKRLAARGVKVRPGMVIGYIVLRGDGPISKRAILAEEFDLRKHKYDAEYYIENQVLPAVLRILEAFGYRKEDLRWQKTKQTGLTAWLNIKKK

SEQ ID NO: 2 - DNA, 2325 bp, synthetic construct
  source 1..2325: mol_type = other DNA
atgattctagacgctgattatataacagaagacggcaaaccgatcatccgcatcttcaagaaggaaaacggtgaatttaaagtggaatacgatcgtaactttcgtccgtatatttatgcgctgctgaaagatgattcgcaaattgacgaagtgcgcaaaattacggccgagcgccacggcaaaatcgtgcgcattatcgacgcagaaaaagtccgtaaaaagtttctgggccgtccgatcgaagtttggcgtttgtacttcgagcacccgcaagatgttccggcaatccgtgataaaatccgcgagcactctgctgtcatcgacatctttgagtatgacattccgtttgcaaaacgttatctgatcgacaaaggtcttatcccgatggaaggagacgaagaactgaagttactggcgtttgcgatcgccactctgtaccatgaaggtgaagagttcgctaagggtccgattattatgatttcctacgcggatgaggaagaagctaaagttatcacttggaaaaagatcgacctgccgtatgttgaggtagtttcctccgaaagagaaatgatcaagcgttttctgaaagtcattcgcgagaaggacccggatgttattatcacctacaatggtgactcgttcgacctgccgtacctggttaagcgggcagaaaagttaggcattaaactcccactgggccgtgatggtagcgaaccgaaaatgcaacgtttgggtgatatgaccgctgtggagattaaaggccgcatccactttgatctgtatcacgtgattcgtcggaccattaacctgccgacctataccttggaggcggtctatgaggcgatcttcggcaaacctaaagagaaggtttatgcgcatgagatcgctgaagcctgggaaaccggtaaaggcttggagcgcgtggcgaagtacagcatggaagatgcgaaggtgacgtacgagctgggtcgtgaattcttcccgatggaggctcagctgtctcgtttggttggtcagccgctgtgggatgtttctcgtagcagcaccggaaacctggtcgagtggtatctgcttcgcaaggcgtatgaacgcaacgagttggcgccaaataaaccggatgaaagagaatacgagcgtcgcttacgtgaaagctatgccggtggttatgttaaggagccggagaagggcctgtgggaaggtctggtcagcctcgacttccgcagcctttatccgtcaattatcatcacgcataacgtgtccccggataccttgaatcgtgaggggtgccgtgaatacgacgtggctccggaggtgggtcataaattctgcaaggattttccgggcttcattccgagcctgctgaagcgtctcttggacgagcgtcaagaaatcaagcggaaaatgaaggcgagcaaagacccgattgaaaagaagatgctggactaccgccaaagagcgattaagatcctggctaatagctactatggttattacggctacgcgaaagcgcgttggtattgtaaagagtgcgcagagagcgttactgcgtggggtcgtgagtacattgaattcgttcgtaaagaattagaggaaaagtttggttttaaggtcctgtacattgacaccgatgggctttacgccaccattccgggcgcaaagccggaggagatcaaaaagaaggcgctggagttcgtggattatatcaacgcaaagctcccgggcttgcttgagctggagtacgagggtttctatgtgcgtggttttttcgtgactaaaaaaaagtatgcgctgatagacgaggagggcaaaatcattacgcgtggcttggagatcgtgcgccgtgactggtctgagatcgcgaaggagacccaggcaaaggtgctggaagccatcctgaaacacggtaatgtggaagaagccgttaagattgtcaaagaggtgaccgaaaagctgagcaaatacgagatcccaccggaaaagcttgttatttatgagcagattacgcgtccactgcacgaatacaaagctatcggtccgcatgttgcggtggccaaacgcttggctgcgcgtggtgttaaggttcgtccgggcatggttatcggctacatcgttttgcgcggtgacggccctatttccaaacgtgcaatcctggcggaagagttcgacctgaggaagcacaaatacgacgccgaatactacatcgagaaccaggtgctgccggcagtactgcgtattctagaggcgtttggctatcgtaaggaggatctgcgttggcagaaaaccaagcagaccggtctgaccgcgtggctgaacattaaaaagaaa